European Patent Application EP 4 631 964 A1, published October 15, 2025. Title: Peptide for cartilage regeneration and uses thereof. Applicant: CAREGEN CO., LTD. The sequence listing filed with the application follows.

SEQUENCE LISTING (16 sequences)

SEQ ID NO: 1 - protein, 10 aa, synthetic construct
RIAFLWVRIK

SEQ ID NO: 2 - protein, 9 aa, synthetic construct
FCRPRNDFF

SEQ ID NO: 3 - DNA, 23 bp, synthetic construct
  source 1..23: mol_type = other DNA
ctatctggacgaagcagctggca

SEQ ID NO: 4 - DNA, 22 bp, synthetic construct
  source 1..22: mol_type = other DNA
atgggtgcaatgtcaatgatgg

SEQ ID NO: 5 - DNA, 20 bp, synthetic construct
  source 1..20: mol_type = other DNA
aactcagggcaggaggatgt

SEQ ID NO: 6 - DNA, 20 bp, synthetic construct
  source 1..20: mol_type = other DNA
tgtccttttggtcgtcgttc

SEQ ID NO: 7 - DNA, 20 bp, synthetic construct
  source 1..20: mol_type = other DNA
ccagcccgaacttgtaaaga

SEQ ID NO: 8 - DNA, 20 bp, synthetic construct
  source 1..20: mol_type = other DNA
tggacgcacaaccatcatac

SEQ ID NO: 9 - DNA, 20 bp, synthetic construct
  source 1..20: mol_type = other DNA
tgagtcctcaagcctcctgt

SEQ ID NO: 10 - DNA, 20 bp, synthetic construct
  source 1..20: mol_type = other DNA
gtgccagatcatcaccacac

SEQ ID NO: 11 - DNA, 20 bp, synthetic construct
  source 1..20: mol_type = other DNA
gcaggctatgagcagtgtga

SEQ ID NO: 12 - DNA, 20 bp, synthetic construct
  source 1..20: mol_type = other DNA
gcatacctcggaagcagaag

SEQ ID NO: 13 - DNA, 20 bp, synthetic construct
  source 1..20: mol_type = other DNA
accacagtccatgccatcac

SEQ ID NO: 14 - DNA, 20 bp, synthetic construct
  source 1..20: mol_type = other DNA
tccaccaccctgttgctgta

SEQ ID NO: 15 - DNA, 20 bp, synthetic construct
  source 1..20: mol_type = other DNA
gcggaggaagtcggtgaaga

SEQ ID NO: 16 - DNA, 20 bp, synthetic construct
  source 1..20: mol_type = other DNA
ccctctcgcttcaggtcagc